European Patent Application EP 4 679 096 A1, published January 14, 2026. Title: Biomarker and analysis method. Applicant: SHIMADZU CORPORATION. Application JP. The sequence listing filed with the application follows.

SEQUENCE LISTING (36 sequences)

SEQ ID NO: 1 - protein, 23 aa, Homo sapiens
RKGPGPGGPGGAGVARGGAGGGP

SEQ ID NO: 2 - protein, 26 aa, Homo sapiens
RKGPGPGGPGGAGVARGGAGGGPSGD

SEQ ID NO: 3 - protein, 28 aa, Homo sapiens
SGERGRKGPGPGGPGGAGVARGGAGGGP

SEQ ID NO: 4 - protein, 32 aa, Homo sapiens
KKIKSGERGRKGPGPGGPGGAGVARGGAGGGP

SEQ ID NO: 5 - protein, 36 aa, Homo sapiens
RKKIKSGERGRKGPGPGGPGGAGVARGGAGGGPSGD

SEQ ID NO: 6 - protein, 24 aa, Homo sapiens
GRKGPGPGGPGGAGVARGGAGGGP

SEQ ID NO: 7 - protein, 25 aa, Homo sapiens
RGRKGPGPGGPGGAGVARGGAGGGP

SEQ ID NO: 8 - protein, 26 aa, Homo sapiens
ERGRKGPGPGGPGGAGVARGGAGGGP

SEQ ID NO: 9 - protein, 23 aa, Homo sapiens
RKKIKSGERGRKGPGPGGPGGAG

SEQ ID NO: 10 - protein, 25 aa, Homo sapiens
ARKKIKSGERGRKGPGPGGPGGAGV

SEQ ID NO: 11 - protein, 29 aa, Homo sapiens
ERGRKGPGPGGPGGAGVARGGAGGGPSGD

SEQ ID NO: 12 - protein, 31 aa, Homo sapiens
KIKSGERGRKGPGPGGPGGAGVARGGAGGGP

SEQ ID NO: 13 - protein, 33 aa, Homo sapiens
RKKIKSGERGRKGPGPGGPGGAGVARGGAGGGP

SEQ ID NO: 14 - protein, 35 aa, Homo sapiens
RKKIKSGERGRKGPGPGGPGGAGVARGGAGGGPSG

SEQ ID NO: 15 - protein, 36 aa, Homo sapiens
ARKKIKSGERGRKGPGPGGPGGAGVARGGAGGGPSG

SEQ ID NO: 16 - protein, 37 aa, Homo sapiens
ARKKIKSGERGRKGPGPGGPGGAGVARGGAGGGPSGD

SEQ ID NO: 17 - protein, 36 aa, Homo sapiens
HMARKKIKSGERGRKGPGPGGPGGAGVARGGAGGGP

SEQ ID NO: 18 - protein, 34 aa, Homo sapiens
FRGHMARKKIKSGERGRKGPGPGGPGGAGVARGG

SEQ ID NO: 19 - protein, 38 aa, Homo sapiens
RGHMARKKIKSGERGRKGPGPGGPGGAGVARGGAGGGP

SEQ ID NO: 20 - protein, 41 aa, Homo sapiens
RGHMARKKIKSGERGRKGPGPGGPGGAGVARGGAGGGPSGD

SEQ ID NO: 21 - protein, 43 aa, Homo sapiens
SFRGHMARKKIKSGERGRKGPGPGGPGGAGVARGGAGGGPSGD

SEQ ID NO: 22 - protein, 43 aa, Homo sapiens
IQASFRGHMARKKIKSGERGRKGPGPGGPGGAGVARGGAGGGP

SEQ ID NO: 23 - protein, 46 aa, Homo sapiens
IQASFRGHMARKKIKSGERGRKGPGPGGPGGAGVARGGAGGGPSGD

SEQ ID NO: 24 - protein, 52 aa, Homo sapiens
PGANAAAAKIQASFRGHMARKKIKSGERGRKGPGPGGPGGAGVARGGAGGGP

SEQ ID NO: 25 - protein, 55 aa, Homo sapiens
PGANAAAAKIQASFRGHMARKKIKSGERGRKGPGPGGPGGAGVARGGAGGGPSGD

SEQ ID NO: 26 - protein, 69 aa, Homo sapiens
NACSKPDDDILDIPLDDPGANAAAAKIQASFRGHMARKKIKSGERGRKGPGPGGPGGAGVARGGAGGGP

SEQ ID NO: 27 - protein, 53 aa, Homo sapiens
DPGANAAAAKIQASFRGHMARKKIKSGERGRKGPGPGGPGGAGVARGGAGGGP

SEQ ID NO: 28 - protein, 75 aa, Homo sapiens
MDCCTENACSKPDDDILDIPLDDPGANAAAAKIQASFRGHMARKKIKSGERGRKGPGPGGPGGAGVARGGAGGGP

SEQ ID NO: 29 - protein, 75 aa, Homo sapiens; identical to SEQ ID NO: 28

SEQ ID NO: 30 - protein, 78 aa, Homo sapiens
MDCCTENACSKPDDDILDIPLDDPGANAAAAKIQASFRGHMARKKIKSGERGRKGPGPGGPGGAGVARGGAGGGPSGD

SEQ ID NO: 31 - protein, 78 aa, Homo sapiens; identical to SEQ ID NO: 30

SEQ ID NO: 32 - protein, 77 aa, Homo sapiens
DCCTENACSKPDDDILDIPLDDPGANAAAAKIQASFRGHMARKKIKSGERGRKGPGPGGPGGAGVARGGAGGGPSGD

SEQ ID NO: 33 - protein, 78 aa, Homo sapiens; identical to SEQ ID NO: 30

SEQ ID NO: 34 - protein, 100 aa, synthetic construct
GSSHHHHHHSSGLVPRGSHMGSMDCCTENACSKPDDDILDIPLDDPGANAAAAKIQASFRGHMARKKIKSGERGRKGPGPGGPGGAGVARGGAGGGPSGD

SEQ ID NO: 35 - protein, 74 aa, Homo sapiens
DCCTENACSKPDDDILDIPLDDPGANAAAAKIQASFRGHMARKKIKSGERGRKGPGPGGPGGAGVARGGAGGGP

SEQ ID NO: 36 - protein, 78 aa, Homo sapiens; identical to SEQ ID NO: 30